European Patent Application EP 4 410 958 A1, published August 7, 2024. Title: Method for producing organoid, medium for producing organoid, organoid and method for evaluating test substance. Applicant: JSR Corporation. Application JP. The sequence listing filed with the application follows.

SEQUENCE LISTING (4 sequences)

SEQ ID NO: 1 - protein, 17 aa, synthetic construct
  CROSSLNK 1..16: note = crosslinked
  VARIANT 2: note = T, W6N, W7N or Nal1, where W6N represents (S)-2-amino-3-(1H-pyrrolo[2,3-c]pyridin-3-yl)propanoic acid, W7N represents (S)-2-amino-3-(1H-pyrrolo[2,3-b]pyridin-3-yl)propanoic acid and Nal1 represents beta-(1-naphthyl)-L-alanine
  VARIANT 4: note = V, K, KCOp or KCOm, where KCOp represents N6-(4-(carboxymethyl)piperazine-1-carbonyl)-L-lysine and KCOm represents N6-(methyl((2S,3R,4R,5R)-2,3,4,5,6-)pentahydroxyhexyl)carbamoyl)-L-lysine
  VARIANT 7: note = T or 4Py, where 4Py represents 4-pyridyl-L-alanine
  VARIANT 9: note = D, F, KCOp, E or KCOm, where KCOp represents N6-(4-(carboxymethyl)piperazine-1-carbonyl)-L-lysine and KCOm represents N6-(methyl((2S,3R,4R,5R)-2,3,4,5,6-)pentahydroxyhexyl)carbamoyl)-L-lysine
  MOD_RES 10: note = N-(2-phenylethyl)-glycine
  MOD_RES 12: note = beta-(1-naphthyl)-L-alanine
  MOD_RES 13: note = T or 4Py, where 4Py represents 4-pyridyl-L-alanine
  VARIANT 15: note = V, E, KCOp or KCOm, where KCOp represents N6-(4-(carboxymethyl)piperazine-1-carbonyl)-L-lysine and KCOm represents N6-(methyl((2S,3R,4R,5R)-2,3,4,5,6-)pentahydroxyhexyl)carbamoyl)-L-lysine
FXVXNVXDXXVXXHXCX

SEQ ID NO: 2 - protein, 4 aa, synthetic construct
NVTD

SEQ ID NO: 3 - protein, 17 aa, synthetic construct
  CROSSLNK 1..16: note = crosslinked
  MOD_RES 2: note = beta-(1-naphthyl)-L-alanine
  MOD_RES 7: note = 4-pyridyl-L-alanine
  MOD_RES 10: note = N-(2-phenylethyl)-glycine
  MOD_RES 12: note = beta-(1-naphthyl)-L-alanine
  MOD_RES 15: note = N6-(4-(carboxymethyl)piperazine-1-carbonyl)-L-lysine
FXVVNVXDDXVXTHXCG

SEQ ID NO: 4 - protein, 17 aa, synthetic construct
  CROSSLNK 1..16: note = crosslinked
  MOD_RES 2: note = beta-(1-naphthyl)-L-alanine
  MOD_RES 10: note = N-(2-phenylethyl)-glycine
  MOD_RES 12: note = beta-(1-naphthyl)-L-alanine
FXVVNVTDDXVXTHVCG